European Patent Application EP 4 800 108 A1, published September 2, 2026. Title: 長期生存型Ｔ細胞、医薬組成物、及び使用方法. Applicant: 慶應義塾. The sequence listing filed with the application follows.

SEQUENCE LISTING (8 sequences)

SEQ ID NO: 1 - RNA, 19 nt, synthetic construct
  source 1..19: mol_type = other RNA
ggatgaacatctacttcta

SEQ ID NO: 2 - RNA, 19 nt, synthetic construct
  source 1..19: mol_type = other RNA
gaatcaatgaagaaatcga

SEQ ID NO: 3 - RNA, 19 nt, synthetic construct
  source 1..19: mol_type = other RNA
ccagataaatctatagcaa

SEQ ID NO: 4 - RNA, 19 nt, synthetic construct
  source 1..19: mol_type = other RNA
gaacatggtaaagaagaga

SEQ ID NO: 5 - RNA, 19 nt, synthetic construct
  source 1..19: mol_type = other RNA
gtaatgcagaagaagacta

SEQ ID NO: 6 - RNA, 19 nt, synthetic construct
  source 1..19: mol_type = other RNA
gctccaaggtgtacgtgaa

SEQ ID NO: 7 - RNA, 19 nt, synthetic construct
  source 1..19: mol_type = other RNA
gctgcttcatctacaaggt

SEQ ID NO: 8 - RNA, 19 nt, synthetic construct
  source 1..19: mol_type = other RNA
gacgtcatcaaggagttca